European Patent Specification EP 3 775 228 B1, published May 6, 2026. Title: ENGINEERED IMMUNE EFFECTOR CELLS AND USE THEREOF. Applicant: FATE THERAPEUTICS, INC. The sequence listing filed with the application follows.

SEQUENCE LISTING (32 sequences)

SEQ ID NO: 1 - DNA, 19 bp, Homo sapiens
  targeting sequence for CD38 Exon 1 knockout (CD38-gNA-1A)
ttgacgcatcgcgccagga

SEQ ID NO: 2 - DNA, 19 bp, Homo sapiens
  targeting sequence for CD38 Exon 1 knockout (CD38-gNA-1B)
attcatcctgagatgaggt

SEQ ID NO: 3 - DNA, 19 bp, Homo sapiens
  targeting sequence for CD38 Exon 1 knockout (CD38-gNA-2A)
actgacgccaagacagagt

SEQ ID NO: 4 - DNA, 19 bp, Homo sapiens
  targeting sequence for CD38 Exon 1 knockout (CD38-gNA-2B)
ctggtcctgatcctcgtcg

SEQ ID NO: 5 - DNA, 19 bp, Homo sapiens
  targeting sequence for CD38 Exon 1 knockout (CD38-gNA-3A)
tcctagagagccggcagca

SEQ ID NO: 6 - DNA, 19 bp, Homo sapiens
  targeting sequence for CD38 Exon 1 knockout (CD38-gNA-3B)
ggagagcccaactctgtct

SEQ ID NO: 7 - protein, 340 aa, Artificial Sequence
  340 a.a. CD64 domain-based construction
MWFLTTLLLWVPVDGQVDTTKAVITLQPPWVSVFQEETVTLHCEVLHLPGSSSTQWFLNGTATQTSTPSYRITSASVNDSGEYRCQRGLSGRSDPIQLEIHRGWLLLQVSSRVFTEGEPLALRCHAWKDKLVYNVLYYRNGKAFKFFHWNSNLTILKTNISHNGTYHCSGMGKHRYTSAGISVTVKELFPAPVLNASVTSPLLEGNLVTLSCETKLLLQRPGLQLYFSFYMGSKTLRGRNTSSEYQILTARREDSGLYWCEAATEDGNVLKRSPELELQVLGLQLPTPVWFHYQVSFCLVMVLLFAVDTGLYFSVKTNIRSSTRDWKDHKFKWRKDPQDK

SEQ ID NO: 8 - protein, 336 aa, Artificial Sequence
  336 a.a. CD64 exon-based construction
MWFLTTLLLWVPVDGQVDTTKAVITLQPPWVSVFQEETVTLHCEVLHLPGSSSTQWFLNGTATQTSTPSYRITSASVNDSGEYRCQRGLSGRSDPIQLEIHRGWLLLQVSSRVFTEGEPLALRCHAWKDKLVYNVLYYRNGKAFKFFHWNSNLTILKTNISHNGTYHCSGMGKHRYTSAGISVTVKELFPAPVLNASVTSPLLEGNLVTLSCETKLLLQRPGLQLYFSFYMGSKTLRGRNTSSEYQILTARREDSGLYWCEAATEDGNVLKRSPELELQVLGLFFPPGYQVSFCLVMVLLFAVDTGLYFSVKTNIRSSTRDWKDHKFKWRKDPQDK

SEQ ID NO: 9 - protein, 335 aa, Artificial Sequence
  335 a.a. CD64 exon-based construction
MWFLTTLLLWVPVDGQVDTTKAVITLQPPWVSVFQEETVTLHCEVLHLPGSSSTQWFLNGTATQTSTPSYRITSASVNDSGEYRCQRGLSGRSDPIQLEIHRGWLLLQVSSRVFTEGEPLALRCHAWKDKLVYNVLYYRNGKAFKFFHWNSNLTILKTNISHNGTYHCSGMGKHRYTSAGISVTVKELFPAPVLNASVTSPLLEGNLVTLSCETKLLLQRPGLQLYFSFYMGSKTLRGRNTSSEYQILTARREDSGLYWCEAATEDGNVLKRSPELELQVLGFFPPGYQVSFCLVMVLLFAVDTGLYFSVKTNIRSSTRDWKDHKFKWRKDPQDK

SEQ ID NO: 10 - DNA, 1032 bp, Artificial Sequence
  exemplifying sequence encoding 340 a.a. CD64 domain-based construction
cttggagacaacatgtggttcttgacaactctgctcctttgggttccagttgatgggcaagtggacaccacaaaggcagtgatcactttgcagcctccatgggtcagcgtgttccaagaggaaaccgtaaccttgcattgtgaggtgctccatctgcctgggagcagctctacacagtggtttctcaatggcacagccactcagacctcgacccccagctacagaatcacctctgccagtgtcaatgacagtggtgaatacaggtgccagagaggtctctcagggcgaagtgaccccatacagctggaaatccacagaggctggctactactgcaggtctccagcagagtcttcacggaaggagaacctctggccttgaggtgtcatgcgtggaaggataagctggtgtacaatgtgctttactatcgaaatggcaaagcctttaagtttttccactggaattctaacctcaccattctgaaaaccaacataagtcacaatggcacctaccattgctcaggcatgggaaagcatcgctacacatcagcaggaatatctgtcactgtgaaagagctatttccagctccagtgctgaatgcatctgtgacatccccactcctggaggggaatctggtcaccctgagctgtgaaacaaagttgctcttgcagaggcctggtttgcagctttacttctccttctacatgggcagcaagaccctgcgaggcaggaacacatcctctgaataccaaatactaactgctagaagagaagactctgggttatactggtgcgaggctgccacagaggatggaaatgtccttaagcgcagccctgagttggagcttcaagtgcttggcctccagttaccaactcctgtctggtttcattaccaagtctctttctgcttggtgatggtactcctttttgcagtggacacaggactatatttctctgtgaagacaaacattcgaagctcaacaagagactggaaggaccataaatttaaatggagaaaggaccctcaagacaaa

SEQ ID NO: 11 - DNA, 1020 bp, ARTIFICIAL SEQUENCE
  exemplifying sequence encoding 336 a.a. CD64 exon-based construction
cttggagacaacatgtggttcttgacaactctgctcctttgggttccagttgatgggcaagtggacaccacaaaggcagtgatcactttgcagcctccatgggtcagcgtgttccaagaggaaaccgtaaccttgcattgtgaggtgctccatctgcctgggagcagctctacacagtggtttctcaatggcacagccactcagacctcgacccccagctacagaatcacctctgccagtgtcaatgacagtggtgaatacaggtgccagagaggtctctcagggcgaagtgaccccatacagctggaaatccacagaggctggctactactgcaggtctccagcagagtcttcacggaaggagaacctctggccttgaggtgtcatgcgtggaaggataagctggtgtacaatgtgctttactatcgaaatggcaaagcctttaagtttttccactggaattctaacctcaccattctgaaaaccaacataagtcacaatggcacctaccattgctcaggcatgggaaagcatcgctacacatcagcaggaatatctgtcactgtgaaagagctatttccagctccagtgctgaatgcatctgtgacatccccactcctggaggggaatctggtcaccctgagctgtgaaacaaagttgctcttgcagaggcctggtttgcagctttacttctccttctacatgggcagcaagaccctgcgaggcaggaacacatcctctgaataccaaatactaactgctagaagagaagactctgggttatactggtgcgaggctgccacagaggatggaaatgtccttaagcgcagccctgagttggagcttcaagtgcttggtttgttctttccacctgggtaccaagtctctttctgcttggtgatggtactcctttttgcagtggacacaggactatatttctctgtgaagacaaacattcgaagctcaacaagagactggaaggaccataaatttaaatggagaaaggaccctcaagacaaa

SEQ ID NO: 12 - DNA, 1005 bp, ARTIFICIAL SEQUENCE
  exemplifying sequence encoding 335 a.a. CD64 exon-based construction
atgtggttcttgacaactctgctcctttgggttccagttgatgggcaagtggacaccacaaaggcagtgatcactttgcagcctccatgggtcagcgtgttccaagaggaaaccgtaaccttgcactgtgaggtgctccatctgcctgggagcagctctacacagtggtttctcaatggcacagccactcagacctcgacccccagctacagaatcacctctgccagtgtcaatgacagtggtgaatacaggtgccagagaggtctctcagggcgaagtgaccccatacagctggaaatccacagaggctggctactactgcaggtctccagcagagtcttcacggaaggagaacctctggccttgaggtgtcatgcgtggaaggataagctggtgtacaatgtgctttactatcgaaatggcaaagcctttaagtttttccactggaactctaacctcaccattctgaaaaccaacataagtcacaatggcacctaccattgctcaggcatgggaaagcatcgctacacatcagcaggaatatctgtcactgtgaaagagctatttccagctccagtgctgaatgcatctgtgacatccccactcctggaggggaatctggtcaccctgagctgtgaaacaaagttgctcttgcagaggcctggtttgcagctttacttctccttctacatgggcagcaagaccctgcgaggcaggaacacatcctctgaataccaaatactaactgctagaagagaagactctgggttatactggtgcgaggctgccacagaggatggaaatgtccttaagcgcagccctgagttggagcttcaagtgcttggcttctttccacctgggtaccaagtctctttctgcttggtgatggtactcctttttgcagtggacacaggactatatttctctgtgaagacaaacattcgaagctcaacaagagactggaaggaccataaatttaaatggagaaaggaccctcaagacaaa

SEQ ID NO: 13 - protein, 153 aa, Artificial Sequence
  153 a.a. CD28 co-stim + CD3-zeta-ITAM
RSKRSRLLHSDYMNMTPRRPGPTRKHYQPYAPPRDFAAYRSRVKFSRSADAPAYQQGQNQLYNELNLGRREEYDVLDKRRGRDPEMGGKPRRKNPQEGLFNELQKDKMAEAFSEIGMKGERRRGKGHDGLFQGLSTATKDTFDALHMQALPPR

SEQ ID NO: 14 - protein, 219 aa, Artificial Sequence
  219 a.a. CD28 hinge + CD28 TM + CD28 co-stim + CD3-zeta-ITAM
IEVMYPPPYLDNEKSNGTIIHVKGKHLCPSPLFPGPSKPFWVLVVVGGVLACYSLLVTVAFIIFWVRSKRSRLLHSDYMNMTPRRPGPTRKHYQPYAPPRDFAAYRSRVKFSRSADAPAYQQGQNQLYNELNLGRREEYDVLDKRRGRDPEMGGKPRRKNPQEGLFNELQKDKMAEAFSEIGMKGERRRGKGHDGLFQGLSTATKDTFDALHMQALPPR

SEQ ID NO: 15 - protein, 263 aa, Artificial Sequence
  263 a.a NKG2D TM + 2B4 + CD3-zeta
SNLFVASWIAVMIIFRIGMAVAIFCCFFFPSWRRKRKEKQSETSPKEFLTIYEDVKDLKTRRNHEQEQTFPGGGSTIYSMIQSQSSAPTSQEPAYTLYSLIQPSRKSGSRKRNHSPSFNSTIYEVIGKSQPKAQNPARLSRKELENFDVYSRVKFSRSADAPAYKQGQNQLYNELNLGRREEYDVLDKRRGRDPEMGGKPRRKNPQEGLYNELQKDKMAEAYSEIGMKGERRRGKGHDGLYQGLSTATKDTYDALHMQALPPR

SEQ ID NO: 16 - protein, 308 aa, Artificial Sequence
  308 a.a CD8 hinge + NKG2D TM + 2B4 + CD3-zeta
TTTPAPRPPTPAPTIASQPLSLRPEACRPAAGGAVHTRGLDFACDSNLFVASWIAVMIIFRIGMAVAIFCCFFFPSWRRKRKEKQSETSPKEFLTIYEDVKDLKTRRNHEQEQTFPGGGSTIYSMIQSQSSAPTSQEPAYTLYSLIQPSRKSGSRKRNHSPSFNSTIYEVIGKSQPKAQNPARLSRKELENFDVYSRVKFSRSADAPAYKQGQNQLYNELNLGRREEYDVLDKRRGRDPEMGGKPRRKNPQEGLYNELQKDKMAEAYSEIGMKGERRRGKGHDGLYQGLSTATKDTYDALHMQALPPR

SEQ ID NO: 17 - protein, 379 aa, Artificial Sequence
  construct mimicking trans-presentation of IL15 (design 3)
MDWTWILFLVAAATRVHSGIHVFILGCFSAGLPKTEANWVNVISDLKKIEDLIQSMHIDATLYTESDVHPSCKVTAMKCFLLELQVISLESGDASIHDTVENLIILANNSLSSNGNVTESGCKECEELEEKNIKEFLQSFVHIVQMFINTSSGGGSGGGGSGGGGSGGGGSGGGSLQITCPPPMSVEHADIWVKSYSLYSRERYICNSGFKRKAGTSSLTECVLNKATNVAHWTTPSLKCIRDPALVHQRPAPPSTVTTAGVTPQPESLSPSGKEPAASSPSSNNTAATTAAIVPGSQLMPSKSPSTGTTEISSHESSHGTPSQTTAKNWELTASASHQPPGVYPQGHSDTTVAISTSTVLLCGLSAVSLLACYLKSRQ

SEQ ID NO: 18 - DNA, 1140 bp, Artificial Sequence
  an exemplary nucleic acid sequence encoding construct mimicking trans-presentation of IL15 (design 3)
atggactggacctggattctgttcctggtcgcggctgcaacgcgagtccatagcggtatccatgtttttattcttgggtgtttttctgctgggctgcctaagaccgaggccaactgggtaaatgtcatcagtgacctcaagaaaatagaagaccttatacaaagcatgcacattgatgctactctctacactgagtcagatgtacatccctcatgcaaagtgacggccatgaaatgtttcctcctcgaacttcaagtcatatctctggaaagtggcgacgcgtccatccacgacacggtcgaaaacctgataatactcgctaataatagtctctcttcaaatggtaacgtaaccgagtcaggttgcaaagagtgcgaagagttggaagaaaaaaacataaaggagttcctgcaaagtttcgtgcacattgtgcagatgttcattaatacctctagcggcggaggatcaggtggcggtggaagcggaggtggaggctccggtggaggaggtagtggcggaggttctcttcaaataacttgtcctccaccgatgtccgtagaacatgcggatatttgggtaaaatcctatagcttgtacagccgagagcggtatatctgcaacagcggcttcaagcggaaggccggcacaagcagcctgaccgagtgcgtgctgaacaaggccaccaacgtggcccactggaccacccctagcctgaagtgcatcagagatcccgccctggtgcatcagcggcctgcccctccaagcacagtgacaacagctggcgtgaccccccagcctgagagcctgagcccttctggaaaagagcctgccgccagcagccccagcagcaacaatactgccgccaccacagccgccatcgtgcctggatctcagctgatgcccagcaagagccctagcaccggcaccaccgagatcagcagccacgagtctagccacggcaccccatctcagaccaccgccaagaactgggagctgacagccagcgcctctcaccagcctccaggcgtgtaccctcagggccacagcgataccacagtggccatcagcacctccaccgtgctgctgtgtggactgagcgccgtgtcactgctggcctgctacctgaagtccagacagtga

SEQ ID NO: 19 - protein, 242 aa, Artificial Sequence
  fused IL15/mb-Sushi construct (design 4)
MDWTWILFLVAAATRVHSGIHVFILGCFSAGLPKTEANWVNVISDLKKIEDLIQSMHIDATLYTESDVHPSCKVTAMKCFLLELQVISLESGDASIHDTVENLIILANNSLSSNGNVTESGCKECEELEEKNIKEFLQSFVHIVQMFINTSSGGGSGGGGSGGGGSGGGGSGGGSLQITCPPPMSVEHADIWVKSYSLYSRERYICNSGFKRKAGTSSLTECVLNKATNVAHWTTPSLKCIR

SEQ ID NO: 20 - DNA, 726 bp, Artificial Sequence
  an exemplary nucleic acid sequence encoding fused IL15/mb-Sushi construct (design 4)
atggactggacctggattctgttcctggtcgcggctgcaacgcgagtccatagcggtatccatgtttttattcttgggtgtttttctgctgggctgcctaagaccgaggccaactgggtaaatgtcatcagtgacctcaagaaaatagaagaccttatacaaagcatgcacattgatgctactctctacactgagtcagatgtacatccctcatgcaaagtgacggccatgaaatgtttcctcctcgaacttcaagtcatatctctggaaagtggcgacgcgtccatccacgacacggtcgaaaacctgataatactcgctaataatagtctctcttcaaatggtaacgtaaccgagtcaggttgcaaagagtgcgaagagttggaagaaaaaaacataaaggagttcctgcaaagtttcgtgcacattgtgcagatgttcattaatacctctagcggcggaggatcaggtggcggtggaagcggaggtggaggctccggtggaggaggtagtggcggaggttctcttcaaataacttgtcctccaccgatgtccgtagaacatgcggatatttgggtaaaatcctatagcttgtacagccgagagcggtatatctgcaacagcggcttcaagcggaaggccggcacaagcagcctgaccgagtgcgtgctgaacaaggccaccaacgtggcccactggaccacccctagcctgaagtgcatcaga

SEQ ID NO: 21 - protein, 375 aa, Artificial Sequence
  protein construct further modified from SEQ ID NO. 17
MDWTWILFLVAAATRVHSGIHVFILGCFSAGLPKTEANWVNVISDLKKIEDLIQSMHIDATLYTESDVHPSCKVTAMKCFLLELQVISLESGDASIHDTVENLIILANNSLSSNGNVTESGCKECEELEEKNIKEFLQSFVHIVQMFINTSSGGGSGGGGSGGGGSGGGGSGGGSLQITCPPPMSVEHADIWVKSYSLYSRERYICNSGFKRKAGTSSLTECVLNKATNVAHWTTPSLKCIRDPALVHQRPAPPSTVTTAGVTPQPESLSPSGKEPAASSPSSNNTAATTAAIVPGSQLMPSKSPSTGTTEISSHESSHGTPSQTTAKNWELTASASHQPPGVYPQGHSDTTVAISTSTVLLCGLSAVSLLACYL

SEQ ID NO: 22 - DNA, 601 bp, Artificial Sequence
  LHA/CD38
cagagggcattgtgtgcacacacgtatagaagcaggcagcccaccctcatgctttccaggaagcaaatgtggctcaggtgtaaagtgcccggttgatgaagggagttagcggagggagtataaggatgtactgtctgcccccttaggacacctgcagaggattaaggtggctgtttctccctggaggtggagtgggtgggtcactgcacaggagcctatagttgttggtcttttaaactcttattggtgtaaccagccacggaactctgaggcaaggggttgggggtgggaagggaaacagagaaaaggcaagtgaaacagaaggggaggtgcagtttcagaacccagccagcctctctcttgctgcctagcctcctgccggcctcatcttcgcccagccaaccccgcctggagccctatggccaactgcgagttcagcccggtgtccggggacaaaccctgctgccggctctctaggagagcccaactctgtcttggcgtcagtatcctggtcctgatcctcgtcgtggtgctcgcggtggtcgtcccgaggtggcgccagcagtggagcggtccgggcaccaccaagcgctttcccgag

SEQ ID NO: 23 - DNA, 252 bp, Artificial Sequence
  insol
tcagcctaaagctttttccccgtatccccccaggtgtctgcaggctcaaagagcagcgagaagcgttcagaggaaagcgatcccgtgccaccttccccgtgcccgggctgtccccgcacgctgccggctcggggatgcggggggagcgccggaccggagcggagccccgggcggctcgctgctgccccctagcgggggagggacgtaattacatccctgggggctttgggggggggctgtccccgtgagctc

SEQ ID NO: 24 - DNA, 1734 bp, Artificial Sequence
  CAG
gttgacattgattattgactagttattaatagtaatcaattacggggtcattagttcatagcccatatatggagttccgcgttacataacttacggtaaatggcccgcctggctgaccgcccaacgacccccgcccattgacgtcaataatgacgtatgttcccatagtaacgccaatagggactttccattgacgtcaatgggtggagtatttacggtaaactgcccacttggcagtacatcaagtgtatcatatgccaagtacgccccctattgacgtcaatgacggtaaatggcccgcctggcattatgcccagtacatgaccttatgggactttcctacttggcagtacatctacgtattagtcatcgctattaccatggtcgaggtgagccccacgttctgcttcactctccccatctcccccccctccccacccccaattttgtatttatttattttttaattattttgtgcagcgatgggggcggggggggggggggggcgcgcgccaggcggggcggggcggggcgaggggcggggcggggcgaggcggagaggtgcggcggcagccaatcagagcggcgcgctccgaaagtttccttttatggcgaggcggcggcggcggcggccctataaaaagcgaagcgcgcggcgggcggggagtcgctgcgacgctgccttcgccccgtgccccgctccgccgccgcctcgcgccgcccgccccggctctgactgaccgcgttactcccacaggtgagcgggcgggacggcccttctcctccgggctgtaattagcgcttggtttaatgacggcttgtttcttttctgtggctgcgtgaaagccttgaggggctccgggagggccctttgtgcggggggagcggctcggggggtgcgtgcgtgtgtgtgtgcgtggggagcgccgcgtgcggctccgcgctgcccggcggctgtgagcgctgcgggcgcggcgcggggctttgtgcgctccgcagtgtgcgcgaggggagcgcggccgggggcggtgccccgcggtgcggggggggctgcgaggggaacaaaggctgcgtgcggggtgtgtgcgtgggggggtgagcagggggtgtgggcgcgtcggtcgggctgcaaccccccctgcacccccctccccgagttgctgagcacggcccggcttcgggtgcggggctccgtacggggcgtggcgcggggctcgccgtgccgggcggggggtggcggcaggtgggggtgccgggcggggcggggccgcctcgggccggggagggctcgggggaggggcgcggcggcccccggagcgccggcggctgtcgaggcgcggcgagccgcagccattgccttttatggtaatcgtgcgagagggcgcagggacttcctttgtcccaaatctgtgcggagccgaaatctgggaggcgccgccgcaccccctctagcgggcgcggggcgaagcggtgcggcgccggcaggaaggaaatgggcggggagggccttcgtgcgtcgccgcgccgccgtccccttctccctctccagcctcggggctgtccgcggggggacggctgccttcgggggggacggggcagggcggggttcggcttctggcgtgtgaccggcggctctagagcctctgctaaccatgttcatgccttcttctttttcctacagctcctgggcaacgtgctggttattgtgctgtctcatcattttggcaaagaatt

SEQ ID NO: 25 - DNA, 1137 bp, Artificial Sequence
  IL15RF(tr)
atggactggacctggattctgttcctggtcgcggctgcaacgcgagtccatagcggtatccatgtttttattcttgggtgtttttctgctgggctgcctaagaccgaggccaactgggtaaatgtcatcagtgacctcaagaaaatagaagaccttatacaaagcatgcacattgatgctactctctacactgagtcagatgtacatccctcatgcaaagtgacggccatgaaatgtttcctcctcgaacttcaagtcatatctctggaaagtggcgacgcgtccatccacgacacggtcgaaaacctgataatactcgctaataatagtctctcttcaaatggtaacgtaaccgagtcaggttgcaaagagtgcgaagagttggaagaaaaaaacataaaggagttcctgcaaagtttcgtgcacattgtgcagatgttcattaatacctctagcggcggaggatcaggtggcggtggaagcggaggtggaggctccggtggaggaggtagtggcggaggttctcttcaaataacttgtcctccaccgatgtccgtagaacatgcggatatttgggtaaaatcctatagcttgtacagccgagagcggtatatctgcaacagcggcttcaagcggaaggccggcacaagcagcctgaccgagtgcgtgctgaacaaggccaccaacgtggcccactggaccacccctagcctgaagtgcatcagagatcccgccctggtgcatcagcggcctgcccctccaagcacagtgacaacagctggcgtgaccccccagcctgagagcctgagcccttctggaaaagagcctgccgccagcagccccagcagcaacaatactgccgccaccacagccgccatcgtgcctggatctcagctgatgcccagcaagagccctagcaccggcaccaccgagatcagcagccacgagtctagccacggcaccccatctcagaccaccgccaagaactgggagctgacagccagcgcctctcaccagcctccaggcgtgtaccctcagggccacagcgataccacagtggccatcagcacctccaccgtgctgctgtgtggactgagcgccgtgtcactgctggcctgctacctgaagtccagacag

SEQ ID NO: 26 - DNA, 66 bp, Artificial Sequence
  P2A
ggatccggagctactaacttcagcctgctgaagcaggctggagacgtggaggagaaccctggacct

SEQ ID NO: 27 - DNA, 765 bp, Artificial Sequence
  hnCD16
atgtggcagctgctgctgcctacagctctcctgctgctggtgtccgccggcatgagaaccgaggatctgcctaaggccgtggtgttcctggaaccccagtggtacagagtgctggaaaaggacagcgtgaccctgaagtgccagggcgcctacagccctgaggacaattccacacagtggtttcacaatgagagcctcatctcaagccaggcctcgagctacttcatcgacgccgccaccgtggacgacagcggcgagtatagatgccagaccaacctgagcaccctgagcgaccccgtgcagctggaagtgcacatcggatggctgctgctgcaggcccccagatgggtgttcaaagaagaggaccccatccacctgagatgccactcttggaagaacaccgccctgcacaaagtgacctacctgcagaacggcaagggcagaaagtacttccaccacaacagcgacttctacatccccaaggccaccctgaaggactccggctcctacttctgcagaggcctcgtgggcagcaagaacgtgtccagcgagacagtgaacatcaccatcacccagggcctggccgtgcctaccatcagcagctttttcccacccggctaccaggtgtccttctgcctcgtgatggtgctgctgttcgccgtggacaccggcctgtacttcagcgtgaaaacaaacatcagaagcagcacccgggactggaaggaccacaagttcaagtggcggaaggacccccaggacaagtga

SEQ ID NO: 28 - DNA, 272 bp, Artificial Sequence
  TKpA
gggggaggctaactgaaacacggaaggagacaataccggaaggaacccgcgctatgacggcaataaaaagacagaataaaacgcacgggtgttgggtcgtttgttcataaacgcggggttcggtcccagggctggcactctgtcgataccccaccgagaccccattggggccaatacgcccgcgtttcttccttttccccaccccaccccccaagttcgggtgaaggcccagggctcgcagccaacgtcggggcggcaggccctgccatagc

SEQ ID NO: 29 - DNA, 600 bp, Artificial Sequence
  RHA/CD38
gatgcgtcaagtacactgaaattcatcctgagatgaggtgggttggcgactaaggcgcaccggtgggcactgcggggacagcagggccccgcgcgcagggaagccgcccggatcgcccggaaccgggcatcttccgtggcgggtcagccgagagcccgccgggtggtgctgagtagggagtcccgggctcggggctccgcgggccgctttcaggagcagctggccttggcaccgagcgtgcccgcgggaggcgggggggggcgctgctcggtggctctgctgcgtagccggtgaacacttggcaccgatgcccgccttctgggcaaggtgccctgagcccagcccctcgccgggctgcagcccaccctcggcgcgctcagcccgcttcaccgcttcagggacggaatagaactcgcagatgcagggtgtcgctgacattttcaactttttctgcggtttccgcccgctgtctctgacccgaaagtgcccccggacggttacagaggacacttaagtggtttgcaaagcctgtggtaggggaggagggtgtagaagggccaaaccacggaacttagttttattcatttatataaagcagca

SEQ ID NO: 30 - DNA, 600 bp, Artificial Sequence
  LHA/CD38
agagggcattgtgtgcacacacgtatagaagcaggcagcccaccctcatgctttccaggaagcaaatgtggctcaggtgtaaagtgcccggttgatgaagggagttagcggagggagtataaggatgtactgtctgcccccttaggacacctgcagaggattaaggtggctgtttctccctggaggtggagtgggtgggtcactgcacaggagcctatagttgttggtcttttaaactcttattggtgtaaccagccacggaactctgaggcaaggggttgggggtgggaagggaaacagagaaaaggcaagtgaaacagaaggggaggtgcagtttcagaacccagccagcctctctcttgctgcctagcctcctgccggcctcatcttcgcccagccaaccccgcctggagccctatggccaactgcgagttcagcccggtgtccggggacaaaccctgctgccggctctctaggagagcccaactctgtcttggcgtcagtatcctggtcctgatcctcgtcgtggtgctcgcggtggtcgtcccgaggtggcgccagcagtggagcggtccgggcaccaccaagcgctttcccgag

SEQ ID NO: 31 - DNA, 63 bp, Artificial Sequence
  T2A
ggcagcggagagggcagaggaagtcttctaacatgcggtgacgtggaggagaatcccggccct

SEQ ID NO: 32 - DNA, 601 bp, Artificial Sequence
  RHA/CD38
cgatgcgtcaagtacactgaaattcatcctgagatgaggtgggttggcgactaaggcgcaccggtgggcactgcggggacagcagggccccgcgcgcagggaagccgcccggatcgcccggaaccgggcatcttccgtggcgggtcagccgagagcccgccgggtggtgctgagtagggagtcccgggctcggggctccgcgggccgctttcaggagcagctggccttggcaccgagcgtgcccgcgggaggcgggggggggcgctgctcggtggctctgctgcgtagccggtgaacacttggcaccgatgcccgccttctgggcaaggtgccctgagcccagcccctcgccgggctgcagcccaccctcggcgcgctcagcccgcttcaccgcttcagggacggaatagaactcgcagatgcagggtgtcgctgacattttcaactttttctgcggtttccgcccgctgtctctgacccgaaagtgcccccggacggttacagaggacacttaagtggtttgcaaagcctgtggtaggggaggagggtgtagaagggccaaaccacggaacttagttttattcatttatataaagcagca